European Patent Application EP 4 538 709 A1, published April 16, 2025. Title: 多发性硬化诊断的标志物及其应用. Applicant: 厦门英博迈生物科技有限公司. The sequence listing filed with the application follows.

SEQUENCE LISTING (21 sequences)

SEQ ID NO: 1 - protein, 613 aa, synthetic construct
MRAPGALLARMSRLLLLLLLKVSASSALGVAPASRNETCLGESCAPTVIQRRGRDAWGPGNSARDVLRARAPREEQGAAFLAGPSWDLPAAPGRDPAAGRGAEASAAGPPGPPTRPPGPWRWKGARGQEPSETLGRGNPTALQLFLQISEEEEKGPRGAGISGRSQEQSVKTVPGASDLFYWPRRAGKLQGSHHKPLSKTANGLAGHEGWTIALPGRALAQNGSLGEGIHEPGGPRRGNSTNRRVRLKNPFYPLTQESYGAYAVMCLSVVIFGTGIIGNLAVMCIVCHNYYMRSISNSLLANLAFWDFLIIFFCLPLVIFHELTKKWLLEDFSCKIVPYIEVASLGVTTFTLCALCIDRFRAATNVQMYYEMIENCSSTTAKLAVIWVGALLLALPEVVLRQLSKEDLGFSGRAPAERCIIKISPDLPDTIYVLALTYDSARLWWYFGCYFCLPTLFTITCSLVTARKIRKAEKACTRGNKRQIQLESQMNCTVVALTILYGFCIIPENICNIVTAYMATGVSQQTMDLLNIISQFLLFFKSCVTPVLLFCLCKPFSRAFMECCCCCCEECIQKSSTVTSDDNDNEYTTELELSPFSTIRREMSTFASVGTHC

SEQ ID NO: 2 - DNA, 1839 bp, synthetic construct
  source 1..1839: mol_type = other DNA
atgcgcgctccgggtgctctgctggcccgtatgagccgcctgctgctgctgttactgctgaaagtgagtgccagcagtgccctgggtgtggcaccggctagccgtaatgaaacctgcctgggtgaaagttgtgccccgaccgttattcagcgccgcggccgtgatgcatggggccctggtaatagcgcccgcgatgttctgcgcgcacgtgcccctcgtgaagaacagggtgccgcatttctggcaggcccgagctgggatctgccggcagcacctggtcgcgatccggctgcaggtcgtggcgcagaagcaagtgccgcaggcccgcctggccctcctacaagaccgcctggcccgtggcgttggaaaggcgcacgtggccaggaaccgagcgaaaccctgggtcgtggtaatccgaccgcactgcagctgtttctgcagattagtgaagaagaagaaaaaggtccgcgcggtgccggtattagtggtcgcagtcaggaacagagcgtgaaaaccgttccgggcgccagtgatctgttttattggccgcgccgtgcaggtaaactgcagggcagtcatcataaaccgctgagcaaaaccgcaaatggtctggcaggtcatgaaggctggaccattgccctgccgggtcgcgcactggcacagaatggtagcctgggtgaaggtattcatgaaccgggtggtccgcgccgtggcaatagcaccaatcgccgcgtgcgcctgaaaaatccgttttatccgctgacccaggaaagctatggcgcatacgctgttatgtgcctgagtgttgttatttttggtacaggcattattggtaatctggcagttatgtgcattgtttgccataattattacatgcgcagtattagcaatagtctgctggccaatctggcattttgggattttctgattattttcttttgcctgccgctggttatttttcatgaactgaccaaaaaatggctgctggaagattttagctgtaaaattgtgccgtatattgaagtggcaagcctgggcgtgaccacctttaccctgtgtgccctgtgtattgatcgttttcgtgcagcaaccaatgttcagatgtattatgaaatgatcgagaattgcagtagtaccaccgcaaaactggccgttatttgggttggcgccctgctgctggcactgccggaagttgttctgcgccagctgagtaaagaagatttgggttttagcggtcgtgccccggcagaacgttgcattattaagattagtccggatctgccggataccatctatgtgctggcactgacctatgatagcgcacgcctgtggtggtattttggttgttatttttgtctgccgaccctgtttaccattacctgtagcctggttaccgcacgtaaaattcgcaaagcagaaaaagcatgcacccgcggcaataagcgtcagattcagctggaaagccagatgaattgtaccgttgttgcactgaccattctgtatggtttttgtattattccggaaaatatctgtaacatcgtgaccgcctatatggcaaccggcgtgagccagcagaccatggatctgctgaatattattagtcagtttctgctgtttttcaagagctgtgttaccccggtgctgctgttttgcctgtgtaaaccgtttagtcgtgcattcatggaatgttgctgttgttgttgtgaagaatgcattcagaaaagtagtaccgttaccagcgatgataatgataatgaatataccaccgaactggaactgagcccgtttagcaccattcgtcgcgaaatgagcacctttgcaagtgtgggcacccattgt

SEQ ID NO: 3 - protein, 265 aa, synthetic construct
MRAPGALLARMSRLLLLLLLKVSASSALGVAPASRNETCLGESCAPTVIQRRGRDAWGPGNSARDVLRARAPREEQGAAFLAGPSWDLPAAPGRDPAAGRGAEASAAGPPGPPTRPPGPWRWKGARGQEPSETLGRGNPTALQLFLQISEEEEKGPRGAGISGRSQEQSVKTVPGASDLFYWPRRAGKLQGSHHKPLSKTANGLAGHEGWTIALPGRALAQNGSLGEGIHEPGGPRRGNSTNRRVRLKNPFYPLTQESYGAYAVM

SEQ ID NO: 4 - DNA, 795 bp, synthetic construct
  source 1..795: mol_type = other DNA
atgcgcgctccgggtgctctgctggcccgtatgagccgcctgctgctgctgttactgctgaaagtgagtgccagcagtgccctgggtgtggcaccggctagccgtaatgaaacctgcctgggtgaaagttgtgccccgaccgttattcagcgccgcggccgtgatgcatggggccctggtaatagcgcccgcgatgttctgcgcgcacgtgcccctcgtgaagaacagggtgccgcatttctggcaggcccgagctgggatctgccggcagcacctggtcgcgatccggctgcaggtcgtggcgcagaagcaagtgccgcaggcccgcctggccctcctacaagaccgcctggcccgtggcgttggaaaggcgcacgtggccaggaaccgagcgaaaccctgggtcgtggtaatccgaccgcactgcagctgtttctgcagattagtgaagaagaagaaaaaggtccgcgcggtgccggtattagtggtcgcagtcaggaacagagcgtgaaaaccgttccgggcgccagtgatctgttttattggccgcgccgtgcaggtaaactgcagggcagtcatcataaaccgctgagcaaaaccgcaaatggtctggcaggtcatgaaggctggaccattgccctgccgggtcgcgcactggcacagaatggtagcctgggtgaaggtattcatgaaccgggtggtccgcgccgtggcaatagcaccaatcgccgcgtgcgcctgaaaaatccgttttatccgctgacccaggaaagctatggcgcatacgctgttatg

SEQ ID NO: 5 - protein, 8 aa, synthetic construct
GFIFSSQA

SEQ ID NO: 6 - protein, 8 aa, synthetic construct
ISSGGSYT

SEQ ID NO: 7 - protein, 18 aa, synthetic construct
ARQRDFGRYYGYDPFFDF

SEQ ID NO: 8 - protein, 7 aa, synthetic construct
SSISSNY

SEQ ID NO: 9 - skipped

SEQ ID NO: 10 - protein, 10 aa, synthetic construct
QQGSSVPRIT

SEQ ID NO: 11 - protein, 123 aa, synthetic construct
EVMLVESGGGLVKPGGSLKLSCAASGFIFSSQAMSWVRQIPEKRLEWVATISSGGSYTYYPDSVKGRFTISRDNAKNTLYLQMSSLTSEDTAMYYCARQRDFGRYYGYDPFFDFWGQGTTLTF

SEQ ID NO: 12 - protein, 107 aa, synthetic construct
EIVLTQSPTTMAASPGEKITITCSASSSISSNYLHWYQQKPGFSPKLLIYRTSNLPSGVPARFSGSGSGTSYSLTIGTMEAEDVATYYCQQGSSVPRITFGAGTKLE

SEQ ID NO: 13 - protein, 8 aa, synthetic construct
GFIFSDYY

SEQ ID NO: 14 - protein, 10 aa, synthetic construct
IRNKAKRYTT

SEQ ID NO: 15 - protein, 12 aa, synthetic construct
ARDTSDYDRFAY

SEQ ID NO: 16 - protein, 11 aa, synthetic construct
QSLVHRNGNTY

SEQ ID NO: 17 - skipped

SEQ ID NO: 18 - protein, 9 aa, synthetic construct
SQSTLLPYT

SEQ ID NO: 19 - protein, 121 aa, synthetic construct
EVKLVESGGGLVQPGGSLRLSCATSGFIFSDYYMSWVRQPPGKALEWLGYIRNKAKRYTTEYNASVKGRFTISRDNSQNILYLQMNTLRAEDSATYYCARDTSDYDRFAYWGQGTLVTVSA

SEQ ID NO: 20 - protein, 112 aa, synthetic construct
DIVMTQTPLSLPVSLGDHASLSCKSSQSLVHRNGNTYLHWFLQKPGQSPKLLIYKVSNRFSGVPDRFSGSGSGTDFTLKISRVEAADLGVYFCSQSTLLPYTFGGGTKLEIK

SEQ ID NO: 21 - protein, 165 aa, synthetic construct
GAEASAAGPPGPPTRPPGPWRWKGARGQEPSETLGRGNPTALQLFLQISEEEEKGPRGAGISGRSQEQSVKTVPGASDLFYWPRRAGKLQGSHHKPLSKTANGLAGHEGWTIALPGRALAQNGSLGEGIHEPGGPRRGNSTNRRVRLKNPFYPLTQESYGAYAVM